European Patent Specification EP 3 938 378 B1, published August 2, 2023. Title: Norovirus-like particles with improved stability. Applicant: Icon Genetics GmbH. The sequence listing filed with the application follows.

SEQUENCE LISTING (61 sequences)

SEQ ID NO: 1 - protein, 544 aa, Norovirus
MMMASKDATPSADGATGAGQLVPEVNTADPIPIDPVAGSSTALATAGQVNLIDPWIINNFVQAPQGEFTISPNNTPGDVLFDLQLGPHLNPFLSHLSQMYNGWVGNMRVRVVLAGNAFTAGKVIICCVPPGFQSRTLSIAQATLFPHVIADVRTLDPVEVPLEDVRNVLYHNNDTQPTMRLLCMLYTPLRTGGASGGTDSFVVAGRVLTCPGPDFNFLFLVPPTVEQKTRPFTVPNIPLKYLSNSRIPNPIEGMSLSPDQTQNVQFQNGRCTIDGQPLGTTPVSVSQLCKFRGRITSGQRVLNLTELDGSPFMAFAAPAPAGFPDLGSCDWHIEMSKIPNSSTQNNPIVTNSVKPNSQQFVPHLSSITLDENVSSGGDYIGTIQWTSPPSDSGGANTNFWKIPDYGSSLAEASQLAPAVYPPGFNEVIVYFMASIPGPNQSGSPNLVPCLLPQEYITHFISEQAPIQGEAALLHYVDPDTNRNLGEFKLYPGGYLTCVPNSSSTGPQQLPLDGVFVFASWVSRFYQLKPVGTAGPARGRLGVRR

SEQ ID NO: 2 - protein, 540 aa, Norovirus
MASKDATPSADGATGAGQLVPEVNTADPIPIDPVAGSSTALATAGQVNLIDPWIINNFVQAPQGEFTISPNNTPGDVLFDLQLGPHLNPFLSHLSQMYNGWVGNMRVRVVLAGNAFTAGKVIICCVPPGFQSRTLSIAQATLFPHVIADVRTLDPVEVPLEDVRNVLYHNNDTQPTMRLLCMLYTPLRTGGASGGTDSFVVAGRVLTCPGPDFNFLFLVPPTVEQKTRPFTVPNIPLKYLSNSRIPNPIEGMSLSPDQTQNVQFQNGRCTIDGQPLGTTPVSVSQLCKFRGRITSGQRVLNLTELDGSPFMAFAAPAPAGFPDLGSCDWHIEMSKIPNSSTQNNPIVTNSVKPNSQQFVPHLSSITLDENVSSGGDYIGTIQWTSPPSDSGGANTNFWKIPDYGSSLAEASQLAPAVYPPGFNEVIVYFMASIPGPNQSGSPNLVPCLLPQEYITHFISEQAPIQGEAALLHYVDPDTNRNLGEFKLYPGGYLTCVPNSSSTGPQQLPLDGVFVFASWVSRFYQLKPVGTAGPARGRLGV

SEQ ID NO: 3 - protein, 540 aa, artificial
  H472R MUTATION
MASKDATPSADGATGAGQLVPEVNTADPIPIDPVAGSSTALATAGQVNLIDPWIINNFVQAPQGEFTISPNNTPGDVLFDLQLGPHLNPFLSHLSQMYNGWVGNMRVRVVLAGNAFTAGKVIICCVPPGFQSRTLSIAQATLFPHVIADVRTLDPVEVPLEDVRNVLYHNNDTQPTMRLLCMLYTPLRTGGASGGTDSFVVAGRVLTCPGPDFNFLFLVPPTVEQKTRPFTVPNIPLKYLSNSRIPNPIEGMSLSPDQTQNVQFQNGRCTIDGQPLGTTPVSVSQLCKFRGRITSGQRVLNLTELDGSPFMAFAAPAPAGFPDLGSCDWHIEMSKIPNSSTQNNPIVTNSVKPNSQQFVPHLSSITLDENVSSGGDYIGTIQWTSPPSDSGGANTNFWKIPDYGSSLAEASQLAPAVYPPGFNEVIVYFMASIPGPNQSGSPNLVPCLLPQEYITHFISEQAPIQGEAALLRYVDPDTNRNLGEFKLYPGGYLTCVPNSSSTGPQQLPLDGVFVFASWVSRFYQLKPVGTAGPARGRLGV

SEQ ID NO: 4 - protein, 540 aa, Artificial Sequence
  T39K, T43D, H472R MUTATIONS
MASKDATPSADGATGAGQLVPEVNTADPIPIDPVAGSSKALADAGQVNLIDPWIINNFVQAPQGEFTISPNNTPGDVLFDLQLGPHLNPFLSHLSQMYNGWVGNMRVRVVLAGNAFTAGKVIICCVPPGFQSRTLSIAQATLFPHVIADVRTLDPVEVPLEDVRNVLYHNNDTQPTMRLLCMLYTPLRTGGASGGTDSFVVAGRVLTCPGPDFNFLFLVPPTVEQKTRPFTVPNIPLKYLSNSRIPNPIEGMSLSPDQTQNVQFQNGRCTIDGQPLGTTPVSVSQLCKFRGRITSGQRVLNLTELDGSPFMAFAAPAPAGFPDLGSCDWHIEMSKIPNSSTQNNPIVTNSVKPNSQQFVPHLSSITLDENVSSGGDYIGTIQWTSPPSDSGGANTNFWKIPDYGSSLAEASQLAPAVYPPGFNEVIVYFMASIPGPNQSGSPNLVPCLLPQEYITHFISEQAPIQGEAALLRYVDPDTNRNLGEFKLYPGGYLTCVPNSSSTGPQQLPLDGVFVFASWVSRFYQLKPVGTAGPARGRLGV

SEQ ID NO: 5 - protein, 540 aa, Artificial Sequence
  T39D, T43K, H472R MUTATIONS
MASKDATPSADGATGAGQLVPEVNTADPIPIDPVAGSSDALAKAGQVNLIDPWIINNFVQAPQGEFTISPNNTPGDVLFDLQLGPHLNPFLSHLSQMYNGWVGNMRVRVVLAGNAFTAGKVIICCVPPGFQSRTLSIAQATLFPHVIADVRTLDPVEVPLEDVRNVLYHNNDTQPTMRLLCMLYTPLRTGGASGGTDSFVVAGRVLTCPGPDFNFLFLVPPTVEQKTRPFTVPNIPLKYLSNSRIPNPIEGMSLSPDQTQNVQFQNGRCTIDGQPLGTTPVSVSQLCKFRGRITSGQRVLNLTELDGSPFMAFAAPAPAGFPDLGSCDWHIEMSKIPNSSTQNNPIVTNSVKPNSQQFVPHLSSITLDENVSSGGDYIGTIQWTSPPSDSGGANTNFWKIPDYGSSLAEASQLAPAVYPPGFNEVIVYFMASIPGPNQSGSPNLVPCLLPQEYITHFISEQAPIQGEAALLRYVDPDTNRNLGEFKLYPGGYLTCVPNSSSTGPQQLPLDGVFVFASWVSRFYQLKPVGTAGPARGRLGV

SEQ ID NO: 6 - protein, 539 aa, Norovirus
MMMASKDAPTSPDGASGAGQLVPEANTAEQISMDPVAGASTAVATAGQVNMIDPWIFNNFVQAPQGEFTISPNNTPGDILFDLQLGPHLNPFLAHLSQMYNGWVGNMRVRILLAGNAFTAGKIIICCVPPGFDARILTIAQATLFPHLIADVRTLEPVELPLEDVRNVLYHNSSQPQPTMRLVAMLYTPLRTGGGSGGTDAFVVAGRVLTCPAPDFSFLFLVPPSVEQKTRVFSVPNIPLKDLSNSRVPVPIQGMFMSPDVNQSVQFQNGRCQIDGQLQGTTPVSLSQLCKIRGKTSSNARVLNLSEVDGTPFIPLESPAPVGFPDLGGCDWHVNFSFQTQDRDPSQSVTFATNDASFVPYLGSVSPHNGEGFQAGDIIGSLGWISAPSDNSQFNVWAIPKYGSSLQMSPILLLLCSPRLWEVILYFYSTFPGSGQPSQLQVPCLLPQEFITHFCNEQAPIAGEAALLHYVDPDTGRNLGEFKLYPDGFMTCVPNSVSSGPQTLPINGVFVFVSWVSRFYQLKPVGTASAARRLGLRRI

SEQ ID NO: 7 - protein, 544 aa, Norovirus
MMMASKDAPTNMDGTSGAGQLVPEANTAEPISMDPVAGAATAVATAGQINMIDPWIMSNFVQAPQGEFTVSPNNTPGDVLFDLQLGPQLNPFLAHLAQMYNGWVGNMRVKVLLAGNAFTAGKIIISCIPPGFTSQNISIAQMTMFPHVIADVRVLEPIEIPLEDVRNVLFHTNDNRPTMRLVCMLYTPLRANGSSSGTDPFVIAGRVLTCPDSNFSFLFLVPPNVEQKTRPFSVPNIPLNTLSNSRVPSLIKSMTISRDQNQIIQFQNGRVTLDGQLQGTTPTSVSQLCKIRGTTYHATGGNGINLTELNGEPYHAFESPAPIGFPDLGGCDWHLTATPTQAFNDGAKVVRLSVTQGAAFAPHLGTIHYTTTDHDYDPNTSIICTLDWLSQTTGQNNVDPWQIPTYGSTLTEAAQLAPPIFPPGFGETLVFFLSDFPISNGKNGLSVPCTLPQEFVTHFVNEQAPIRGEAALLHYVDPDTHRNLGEFKLYPEGFMTCVPNTSGGGPQTLPINGVFVFVSWVSRFYQLKPVGTAGAARRLGIRRS

SEQ ID NO: 8 - protein, 545 aa, Norovirus
MMMASKDAPTNMDGTSGAGQLVPEANTAEPISMEPVAGAATAAATAGQVNMIDPWIMNNYVQAPQGEFTISPNNTPGDILFDLQLGPHLNPFLSHLAQMYNGWVGNMKVKVLLAGNAFTAGKIIISCIPPGFAAQNISIAQATMFPHVIADVRVLEPIEIPLEDVRNVLFHNNDNTPTMRLVCMLYTPLRASGSSSGTDPFVIAGRVLTCPSPDFSFLFLVPPNVEQKTKPFSVPNLPLNILSSSRVPSLIKSMMISRDHGQMVQFQNGRVTLDGQLQGTTPTSASQLCKIRGSVFHANGGNGYNLTELDGSPYHAFESPAPIGFPDLGECDWHMEASPTIQFDTGDVIKQINVKQESAFAPHLGTVQADGLDGVSANTNMIAKLGWVSPVSDGHRRDVDPWVIPRYGSTLTEAAQLAPPIYPPGFGEAIVFFMSDFPIAHGTNGLSVPCTIPQEFVTHFVNEQAPTRGEAALLHYLDPDTHRNLGEFKLYPDGFMTCVPNSSGSGPQTLPINGVFVFVSWVSRFYQLKPVGTAGPARRLGIRRS

SEQ ID NO: 9 - protein, 545 aa, Norovirus
MMMASKDAPSNMDGTSGAGQLVPEANTAEPINMESVVGAATATATAGQVNLIDPWIMNNYVQAPQGEFTISPNNTPGDVLFDLQLGPHLNPFLSHLSRMYNGWVGNMKVRVMLAGNAFSAGKIIICCIPPGFTSQSISIAQATMFPHVIADVRVLEPIDVPLDDVRNVLFHNNDNAQTMRLLCMLYTPLRTGASSSGSDPFVIAGRVLTCPTQDFNFLFLVPPDVEQKTKPFSVPNIPLNLMSNSRVPALIDGMTVSSDQNQVVQFQNGRVTLDGQLQGTTAVSASCVAKIRGRIFSNASHYGINLTEVDGTQYHAFDSPAPLGFPDFGNCDWHVTGTKASQGDLQTDNPTISGTIKSYESSFAPHLGTVRIEGDDNELARFNGKDVLLNLTWFSQRNGSQLNLWTIPSYGSNLTEASQLAPPIYPPGFGEAIVYFTSTFPAISRPSVPCTMPQEFVSHFVNEQAPTRGEAALLHYLDPDTHRNLGEFKMYPEGFFTCVPNAGGSGPQTLPINGVFVFVSWVSRYYQLKPVGTVGMTRRLGLMKQ

SEQ ID NO: 10 - protein, 530 aa, Norovirus
MMMASKDATSSVDGASGAGQLVPEVNASDPLAMDPVAGSSTAVATAGQVNPIDPWIINNFVQAPQGEFTISPNNTPGDVLFDLSLGPHLNPFLLHLSQMYNGWVGNMRVRIMLAGNAFTAGKIIVSCIPPGFGSHNLTIAQATLFPHVIADVRTLDPIEVPLEDVRNVLFHNNDRNQQTMRLVCMLYTPLRTGGGTGDSFVVAGRVMTCPSPDFNFLFLVPPTVEQKTRPFTLPNLPLSSLSNSRAPLPISSMGISPDNVQSVQFQNGRCTLDGRLVGTTPVSLSHVAKIRGTSNGTVINLTELDGTPFHPFEGPAPIGFPDLGGCDWHINMTQFGHSSQTQYDVDTTPDTFVPHLGSIQANGIGSGNYVGVLSWISPPSHPSGSQVDLWKIPNYGSSITEATHLAPSVYPPGFGEVLVFFMSKMPGPGAYNLPCLLPQEYISHLASEQAPTVGEAALLHYVDPDTGRNLGEFKAYPDGFLTCVPNGASSGPQQLPINGVFVFVSWVSRFYQLKPVGTASSARGRLGLRR

SEQ ID NO: 11 - protein, 546 aa, Norovirus
MMMASKDAPQSADGASGAGQLVPEVNTADPLPMEPVAGPTTAVATAGQVNMIDPWIVNNFVQSPQGEFTISPNNTPGDILFDLQLGPHLNPFLSHLSQMYNGWVGNMRVRILLAGNAFSAGKIIVCCVPPGFTSSSLTIAQATLFPHVIADVRTLEPIEMPLEDVRNVLYHTNDNQPTMRLVCMLYTPLRTGGGSGSSDSFVVAGRVLTAPSSDFSFLFLVPPTIEQKTRAFTVPNIPLQTLSNSRFPSLIQGMILSPDASQVVQFQNGRCLIDGQLLGTTPATSGQLFRVRGKINQGARTLNLTEVDGKPFMAFDSPAPVGFPDFGKCDWHMRISKTPNNTSSGDPMRSVSVQTNVQGFVPHLGSIQFDEVFNHPTGDYIGTIEWISQPSTPPGTDINLWEIPDYGSSLSQAANLAPPVFPPGFGEALVYFVSAFPGPNNRSAPNDVPCLLPQEYITHFVSEQAPTMGDAALLHYVDPDTNRNLGEFKLYPGGYLTCVPNGVGAGPQQLPLNGVFLFVSWVSRFYQLKPVGTASTARGRLGVRRI

SEQ ID NO: 12 - protein, 544 aa, Norovirus
MMMASKDAPTNMDGTSGAGQLVPEANTAEPISMEPVAGAATAAATAGQVNMIDPWIMNNYVQAPQGEFTISPNNTPGDILFDLQLGPHLNPFLSHLAQMYNGWVGNMKVKVLLAGNAFTAGKIIISCIPPGFASQNISIAQATMFPHVIADVRVLEPIEVPLEDVRNVLFHNNDNTPTMRLVCMLYTPLRASGSSSGTDPFVIAGRVLTCPSPDFSFLFLVPPNVEQKTKPFSVPNLPLNVLSNSRVPSLIKSMMVSQDHGQMVQFQNGRVTLDGQLQGTTPTSASQLCKMRGTVYHASGGQGLNLTEIDGTPYHAFESPAPIGFPDIGDSDWHINASPATTFDSGESIKRLDMEQGSSFAPHLGTVHYTNADYPANTDLICSLEWLSPPSGGTPNKVNPWTIPRYGSTLTEAAQLAPPIYPPGFGEAIVFFMSDFPIANGQDGLKVPCTIPQEFVTHFVNEQAPTRGEAALLHYVDPDTHRNLGEFKLYPEGFMTCVPNSSGSGPQTLPINGVFTFVSWVSRFYQLKPVGTTGPVRRLGIRRS

SEQ ID NO: 13 - protein, 544 aa, Norovirus
MMMASKDAPTNMDGTSGAGQLVPEANTAEPISMEPVAGAATAAATAGQVNMIDPWIMNNYVQAPQGEFTISPNNTPGDILFDLQLGPHLNPFLSHLAQMYNGWVGNMKVKVLLAGNAFTAGKIIISCIPPGFASQNISIAQATMFPHVIADVRVLEPIEVPLEDVRNVLFHNNDNSPTMRLVCMLYTPLRASGSSSGTDPFVIAGRVLTCPSPDFSFLFLVPPNVEQKTKPFSVPNLPLNTLSNSRVPSLINAMMISRDHGQMVQFQNGRVTLDGQLQGTTPTSLSQLCKIRGKVFLASGGNGLNLTELDGSAYHAFESPAPIGFPDIGDCDWHMNATATSNFTGSNDEHQILVKQESTFAPHLGHVQADHLPEVANTDLMVSLSWISPVSDQHRRDVDPWVIPRYGSTLTEAAQLAPPIYPPGFGEAIVFFMSDFPVVSGVNGMRIPCTLPQEYVAHFVNEQAPTRGEAALLHYVDPDTHRNLGEFKIYPEGFMTCVPNSSGTGPQTLPINGVFTFVSWVSRFYQLKPVGTAGPARRLGIRRS

SEQ ID NO: 14 - protein, 533 aa, Norovirus
MMMASKDATPSADGATGAGQLVPEVNTADPIPIDPVAGSSTALATAGQVNLIDPWIINNFVQAPQGEFTISPNNTPGDVLFDLQLGPHLNPFLSHLSQMYNGWVGNMRVRVVLAGNAFTAGKVIICCVPPGFQSRTLSIAQATLFPHVIADVRTLDPVEVPLEDVRNVLYHNNDTQPTMRLLCMLYTPLRTGGASGGTDSFVVAGRVLTCPGPDFNFLFLVPPTVEQKTRPFTVPNIPLKYLSNSRIPNPIEGMSLSPDQTQNVQFQNGRCTIDGQPLGTTPVSVSQLCKFRGRITSGQRVLNLTELDGSPFMAFAAPAPAGFPDLGSCDWHIEMSKIPNSSTQNNPIVVNSVKPNSQQFVPHLSSITLDDNVSSGGDYIGTIQWTSPPSDSGGANTNFWKIPDYGSSLAEASQLAPAVYPPGFNEVIVYFMASIPGPNQSGSPNLVPCLLPQEYITHFISEQAPIQGEAALLHYVDPDTNRNLGEFKLYPGGYLTCVPNSSSTGPQQLPLDGVFVFASWVSRFYQLKPVGTA

SEQ ID NO: 15 - protein, 544 aa, Norovirus
MMMASKDATPSADGATGAGQLVPEVNTADPIPIDPVAGSSTALATAGQVNLIDPWIINNFVQAPQGEFTISPNNTPGDVLFDLQLGPHLNPFLSHLSQMYNGWVGNMRVRVVLAGNAFTAGKVIICCVPPGFQSRTLSIAQATLFPHVIADVRTLDPVEVPLEDVRNVLYHNNDTQPTMRLLCMLYTPLRTGGASGGTDSFVVAGRVLTCPGPDFNFLFLVPPTVEQKTRPFTVPNIPLKYLSNSRIPNPIEGMSLSPDQTQNVQFQNGRCTIDGQPLGTTPVSVSQLCKFRGRITSGQRVLNLTELDGSPFMGFGAPAPAGFPDLGSCDWHIEMSKIPNSSTQNNPIVTNSVKPNSQQFVPHLSSITLDENVSSGGDYIGTIQWTSPPSDSGGANTNFWKIPDYGSSLAEASQLAPAVYPPGFNEVIVYFMASIPGPNQSGSPNLVPCLLPQEYITHFISEQAPIQGEAALLHYVDPDTNRNLGEFKLYPGGYLTCVPNSSSTGPQQLPLDGVFVFASWVSRFYQLKPVGTAGPARGRLGVRR

SEQ ID NO: 16 - protein, 543 aa, Norovirus
MMMASKDATPSADGANGAGQLVPEVNNAEPLPLDPVAGASTALATAGQVNMIDPWIFNNFVQAPQGEFTISPNNTPGDILFDLQLGPHLNPFLAHLSQMYNGWVGNMRVRVILAGNAFTAGKVIICCVPPGFQSRTLSIAQATLFPHIIADVRTLEPIEIPLEDVRNTLYHTNDNQPTMRLLCMLYTPLRTGGGSGGTDAFVVAGRVLTSPSPDFNFLFLVPPTVEQKTRPFSVPNIPLQLLSNSRVPNLIQSMVPSPDQAQNVQFQNGRCTTDGQLLGTTPVSVSQILKFRGKVSAGSKVINLTELDGSPFLAFEAPAPTGFPDLGTSDWHIEMSLNSNSQSSGNPILLRDIQPNSSDFVPHLGSVAVTTAIDTAGDYTGTIQWTSQPSNVTPVPDVNFWTIPQYGSNLAEASQLAPVVYPPGFGEAIVYFMSPIPGPNTAHKPNLVPCLLPQEFVTHFVSEQAPSMGEAALVHYVDPDTNRNLGEFKLYPEGFITCVPNGTGPQQLPLNGVFVFASWVSRFYQLKPVGTANSARGRLGVRR

SEQ ID NO: 17 - protein, 541 aa, Norovirus
MMMASKDATPSADGANGAGQLVPEVNNAEPLPLDPVAGASTALATAGQVNMIDPWIFNNFVQAPQGEFTISPNNTPGDILFDLQLGPHLNPFLAHLSQMYNGWVGNMRVRVILAGNAFTAGKVIICCVPPGFQSRTLSIAQATLFPHVIADVRTLEPLEIPLEDVRNTLYHNNDSQPTMRLLCMLYTPLRTGGGSGGTDAFVVAGRVLTCPSPDFNFLFLVPPTVEQKTRPFSVPNIPLQNLSNSRVPSLIQSMVLSSDHAQTVQFQNGRCTTDGHLLGTTPVSSGQLMKFRGKVTPGSKVLNLTELDGSPFLAFEPPAPAGFPDLGKCDWHIEMSLYQVNNQDNPIVLRAIEPNSSSFVPHLGSVSFNQNVDAAGDYVCTIQYTSPPSNSHDADVDFWSIPDYGSNLAEASQLAPVVYPPGFGEAIVYFMSRVPGWNRTNRLNLVPCLLPQEFIGHFVSEQAPAIGEAALLHYVDPDTNRNLGEFKLYPEGFITCVPNGTGPQQLPLNGVFVFSSWVSRFYQLKPVGTASSARGRLGIRR

SEQ ID NO: 18 - protein, 540 aa, Norovirus
MMMASKDVPTSPDGASGAGQLVPEVNTADQISMDPVAGASTAVATAGQVNMIDPWIFNNFVQAPQGEFTISPNNTPGDILFDLQLGPHLNPFLAHLSQMYNGWVGNMRVRILLAGNAFTAGKIIICCVPPGFDARILTIAQATLFPHLIADVRTLEPVELPLEDVRNVLYHNSSQPQPTMRLVAMLYTPLRTGGGSGGTDAFVVAGRVLTCPAPDFSFLFLVPPSVEQKTRVFSVPNIPLKDLSNSRVPTLIQGMFVSPDVNQSVQFQNGRCQIDGQLQGTTPVSLSQLCKIRGKTSSNTRVLNLSEVDGTPFVPLESPAPVGFPDIGGCDWHVGFTFEARDQGPSQNVTFATNDSSFVPYLGSISPHNGDGFHSGDIIGSLDWISAPSDGSALDVWSIPKYGSSLPDVTHLAPAVFPPGFGEVILYFHSKFPGSGPTDKLRVPCLMPQEFITHFCDEQAPIAGEAALLHYVDPDAGRNLGEFKLYPDGFMTCVPNSISSGPQTLPINGVFVFVSWVSRFYQLKPVGTASMARRLGLRRI

SEQ ID NO: 19 - protein, 539 aa, Norovirus
MMMASKDAPSNMDGTSGAGQLVPEVNAAEPLPLEPVVGAATAVATAGQVNLIDPWIMNNFVQAPEGEFTISPNNTPGDILFDLQLGPHLNPFLQHLSQMYNGWVGNMRVRVMLAGNAFTAGKIIICCVPPGFASQNISIGQATMFPHVIADVRVLEPIEIPLDDVRNVLFHTNESRPTMRLLCMLYTPLRAGGASSGTDPFVIAGRVLTCPSPDFNFLFLVPPSVEQKTRQLTVPNIPLNNLANSRVPAMINKMTVSTDQSQVVQFQNGRCTLEGQLLGTTPVSASQVARIRGKVFSTASGKGLNLTELDGTPYHAFESPAPLGFPDIGACDWHVSTFKVDQNLSGDPMSRLDIKQNAPFAPHLGSIEFTSDQEPTGDQLGTLAWVSPSTSGARVDPWKIPSYGSTVTESTHLAPPIFPPGFGEAIVYFMSDFPIVSGNTAQVPCTLPQEFVSHFVEQQAPIRGEAALLHYVDPDTHRNLGEFKLYPDGFITCVPNTGGGPQNLPINGVFVFSSWVSRYYQLKPVGTAGPARRLGVRRV

SEQ ID NO: 20 - protein, 543 aa, Norovirus
MMMASKDAPTNMDGTSGAGQLVPEANTAEPLPIKPVAGAATAVATAGQVNMIDPWIMNNFVQAPQGEFTISPNNTPGDILFDLQLGPHLNPFLAHLSRMYNGWVGNMQVRIMLAGNAFSAGKIIVCCIPPGFSSQSISIAQATMFPHVIADVRVLEPIDVPLDDVRNVLFHNNDNPQTMRLLCMLYTPLRSGGTSSGTDPFVIAGRVLTCPTPDFSFLFLVPPDIEQRTKPFSVPNIPMNLMSNSRVSMLIDGMMVSNDQNQVPQFQNGRVTLDGQLQGTTTVSAACVARMRGRIFNNNGNYGVNLTELDGNPYHAFDSPAPLGFPDFGNCDLHMTFVKINPNELSSGDPSGKVVIRSYDATFAPHLGTVKLENDDELARFVGKEVVLELTWVSNREGATLNLWAVPNYGSSLTQASQLAPPIYPPGFGEAIVYFTSTFPTVSNPKVPCTLPQEFVSHFVNEQAPTRGDAALLHYVDPDTHRNLGEFKMYPEGYMTCVPNAGGGPQTLPINGVFVFISWVSRYYQLKPVGTAGAARRLGLRRS

SEQ ID NO: 21 - protein, 550 aa, Norovirus
MMMASKDATSNMDGTSGAGQLVPENNNTSEPINMEPVAGAVTAAATAGQVNMIDPWIMNNYVQAPQGEFTISPNNTPGDILFDLQLGPHLNPFLAHLSQMYNGWVGNMKVRVVLAGNAFSAGKIIVCCIPPGFSAPNISIAQATMFPHVIADVRVLEPIDIPLDDVRNVLFHNNDNGNQTMRLLCMLYTPLRSGGTSSGTDPFVIAGRVLTCPTPDFNFLFLVPPTVEQKTKQFSVPNLPLNVMSNSRVPSLLNAMVVSPDQAQVVQFQNGRCTLDGQMLGTTTVSASCVARFRGKTFQAPDNRLGINLAEISGEPYHAFESPAPLGFPDFGDGDWHVTATKVTPSQLEANDPVVMGNVQPYNPQFAPHLGTLVVENPTPDNVTTGTDLLFNITWLSNRANNRFNPWVIPNYGSTLTEAAQLAPSIFPPGFGETIVYFNSTFPAVGATTHAAIPCLLPQEFVAHFVNEQAPIRGEAALLHYIDPDTHRNLGEFKIYPEGFVTCVPNVGGTGPQSLPTNGIFVFVSWVSRYYQLKPVGTAGQARRLGFRRV

SEQ ID NO: 22 - protein, 538 aa, Norovirus
MKMASNDANPSDGSAANLVPEVNNEVMALEPVVGAAIAAPVAGQQNVIDPWIRNNFVQAPGGEFTVSPRNAPGEILWSMPLSPELNPYLSHLSRMYNGYAGGFEVQVILAGNAFTAGKIIFAAIPPNFPTDGLSPSQVTMFPHIIVDVRQLEPVLIPLPDVRNNFYHYNQANDSTLKLIAMLYTPLRANNAGDDVFTVSCRVLTRPSPDFDFIFLVPPTVESRTKPFTVPILTVDEMTNSRFPTPLEKLHTGPNNSIVVQPQNGRCTIDGVLLGTTQLSTVNICNFRGSTTRAGQSHAYTMNLVSQNWNNYDPTEEIPAPLGTPDFVGKIVGMLSQTTRENSSTRAHKATVSTGDAHFTPKSGSVLFTTDTDDLQNGQNTRFTPVGVAQDGEPHQNEPQQWRLPNYSGTPGHNVHLAPPVAPTFPGEQLLFFRSTMPGCGGYPNMDLDCLLPQEWVRHFYQEAAPAQSDVALLRFVNPDTGRVLFECKLHKAGYITVSHTGPYDLVIPPNGYFRFDSWVNQFYALAPMGTGTGRRRAL

SEQ ID NO: 23 - protein, 543 aa, Norovirus
MKMASNDAAPSNDGAAGLVPEINNETMALEPVAGGAIAAPLTGQTNFIDPWIRNNYVQAPNGEFTVSPRNSPGEILLNLELGPELNPFLAHLSRMYNGYAGGIDVQVIMAGNAFTAGKIIFAAVPPHFPIDNISPPQITMFPHIIIDVRTLEPVNIPLPDVRNSFFHYSQNNEPRMRLLAMLYTPLRSNGSADDVFTVSCRVLTKPSADFEFNYLVPPTVESRTKPFTIPILTIGEMTNSRFPVAIDMLHTSPTDNFIVQPQNGRCTLDGELQGTTQLVTSNICAFRGSISGHENNGDQHQWHFSITNPNGTPFDPTEDVPAPLGTPDFKGQLYGVISQRNREGSPGNGNQKANRSHEGVISTVAPRFTPKLGSVMIGTWTTDDIQDQPSRFTPVGLNDDDNYKQWELPNYSGALTLNMGLAPSVFPTYPGEQLLFFRSYIPMKGGYGSPYIDCLIPQEWISHFYQESAPSQTDVALIRYVNPDTGRVLFEAKLHRQGYITVAKTGDSPINVPANGYFRFDSWVSQFYSLAPMGTGNGRRRIQ

SEQ ID NO: 24 - protein, 555 aa, Norovirus
MRMASSDAPVSGTDGAAGLVPESQQEVLPLEPVAGVQLAAPVAGQSNIIDPWIRMNFVQAPAGEFTVSPRNAPGEVLIDLELGPELNPYLNHLARMYNGYVGGMEVEVVLAGNAFTAGKILFAAVPPSFPTHGISAAQATMLPHVIVDVRQLEPVRLPLPDVRNVMFHFCQENKEPRMRIVAILYTPLRANGAGDDVFTVSCRVLTRPSPDFDFIFLVPPSVESKLKQFTLPNLQPNEMTNSRFPTGITQLYTSPNTNLVVQFQNGRCLLDGTLLGTTPVRAADICSFRGVTSTEVDATDSPRVAGSHRIMVQLKEPDGEEFSPTGPNPAPVGTPDFQAAIFGTLSQRNTGGTGQNSNRAHFAYFYTRNPTFAPGIGTVVFSFDTTDFQNRQPTKFSPSGVFDDDSSEPFNQFSLPYYNGSLGAVDAGKLAPPVAPNYPGEQILYFRGNIPFKGGYGEGEIDSLLPQEWITHFYAEQAPTQGDAALLRYYNPDTGRVLFECKLHREGFITINYTGSNALAVPVNGVFRFEGWVNKFYTLTPMGNGNGRRGRRREL

SEQ ID NO: 25 - protein, 535 aa, Norovirus
MKMASNDANPSSDGSANLVPEISNEVMALEPVAGAAIAAPVAGQQNIIDPWIRNNFVQAPGGEFTVSPRNAPGEVLLNLPLSPDINPYLAHLSRMYNGYAGGVEVEVVLAGNAFTAGKIIFAAVPPNFPPENLSPSQITMLPHIIVDVRQLEPVRIPLPDVRNNFYHYSRENDSTLRLIAMLYTPLRANNAGDDVFTVSCRVLTRPSPDFDFIFLVPPTVESKSKPFTIPMLTIEEMTNSRFPAPLELMTTGPSHDIVVQPQNGRCTIDGVLLGTTQLSPVNICSLRGVPTKRTNGNDNCFVQLENPNGSAYDPTEDIPAVLGSPDFVGELYGTITQRSSDNSTRAHPFTLNTGSPRYTPKIGSVDIRVTDVSDLQDHDPVKLTPVGLSGDRGSIHQWQLPNYSGVATHNMHLAPSVAPLFPGEQILFFRSTVPGCGGYPNSNIDCLIPQEWVQHFYQEGAPARTDVALLRFINPDTGRVLFECKLHKHGFITVAYSGNHDLVMPPNGYFRFESWVNQFHTLAPMGTGSGRRRIQ

SEQ ID NO: 26 - protein, 555 aa, Norovirus
MKMASKDASPSTDGTANLVPESQQEVLALQPVAGAQIAAPVAGQFNVIDPWIYQNFVQAPEGEFTVSPRNSTGEILMNLELGPQLNPYLAHLARMYNAYAGGFEVQVLLAGNAFTAGKIIVCAVPPNFPLQNISAAQATQLPHVVVDVRQLEPVVLPLPDVRAGFYHYNQVEESRMRLVAILYTPLRTNSAGDDAFTVSCRILTRPAPDFSFFFLIPPTIESKTTPFTLPRLPISEMTNSRFPLVIKGMVVDPNLPLQANFQNGRITLDGELQGTTLPTSTSIGRISGTHMSSTPSRIIQHEDSGDSTQPRVFNPVWMDLTENNWTEFQPFNDQPAPLGCPDFKAKILGTLIRQPNNGSYYFDAYLDTRQHGTFAPYTGHAAVHSDQQAGHLAQGYKIQFSPTGIESDQNTDLNQLPDYGGAMTVSKGLAPAAAPDFPGEMILYFVSDMPVRNPNGERRDTEILCLLPQEMVTHFYEQQAPSQGDVALVRYINAETGRVMFEGKLHRNGFFTVSATARTLIVPDGYFRFDSWVNRFYTLSPMGTGNGRRRARMLE

SEQ ID NO: 27 - protein, 535 aa, Norovirus
MKMASNDVAPSNDGAAGLVPEVSNETMALEPVAGASIAAPLTGQNNVIDPWIRMNFVQAPNGEFTVSPRNSPGEVLLNLELGPELNPFLAHLARMYNGYAGGVEVQVLLAGNAFTAGKLVFAAIPPHFPLENLSPGQITMFPHVIIDVRTLEPVLLPLPDVRNNFFHYNQQPEPRMRLVAMLYTPLRSNGSGDDVFTVSCRVLTRPSPDFDFNYLVPPTVESKTKPFTLPILTIGELSNSRFPVPIDELYTSPNEGVVVQPQNGRSTLDGELLGTTQLVPSNICALRGRINAQVPDDHHQWNLQVTNANGTSFDPTEDVPAPLGTPDFLANIYGVTSQRNPDNTCRAHDGVLATWSPKFTPKLGSVVLGTWEESDLDLNQPTRFTPVGLYDTNHFDQWILPNYSGRLTLNMNLAPSVAPLFPGEQILFFRSHIPLKGGTSNGAIDCLLPQEWIQHFYQESAPSPTDVALIRYTNPDTGRVLFEAKLHRQGFITVANSGSRPIVVPPNGYFRFDSWVNQFYSLAPMGTGNGRRRVQ

SEQ ID NO: 28 - protein, 542 aa, Norovirus
MKMASIDAAPSTDGAAGLVPESNNEVMALEPVAGAALAAPVTGQTNIIDPWIRANFVQAPNGEFTVSPRNAPGEVLLNLELGPELNPYLAHLARMYNGYAGGMEVQVMLAGNAFTAGKLVFAAVPPHFPVENLSPQQITMFPHVIIDVRTLEPVLLPLPDVRNNFFHYNQKDDPKMRIVAMLYTPLRSNGSGDDVFTVSCRVLTRPSPDFDFTYLVPPTVESKTKPFTLPILTLGELSNSRFPVSIDQMYTSPNEVISVQCQNGRCTLDGELQGTTQLQVSGICAFKGEVTAHLHDNDHLYNVTITNLNGSPFDPSEDIPAPLGVPDFQGRVFGVISQRDKHNSPGHNEPANRGHDAVVPTYTSQYTPKLGQIQIGTWQTDDLTVNQPVKFTPVGLNDTEHFNQWVVPRYAGALNLNTNLAPSVAPVFPGERLLFFRSYIPLKGGYGNPAIDCLLPQEWVQHFYQEAAPSMSEVALVRYINPDTGRALFEAKLHRAGFMTVSSNTSAPVVVPANGYFRFDSWVNQFYSLAPMGTGNGRRRVQ

SEQ ID NO: 29 - protein, 542 aa, Norovirus
MKMASNDAAPSNDGAAGLVPEINNETMALEPVAGGAIAAPLTGQTNFIDPWIRGNYVQAPNGEFTVSPRNSPGEILLNLELGPELNPFLAHLSRMYNGYAGGIDVQVIMAGNAFTAGKIIFAAVPPHFPVENISPPQITMFPHIIVDVRTLEPINIPVPDVRNNFFHYNQDRDSRMRLVAMLYTPLRSNGSTDDVFTVSCRVLTKPSADFEFNYLVPPTVESRTKPFSIPILTIGEMTNSRFPLPIDMLYTSPTENLVVQPQNGRCTTEGELLGTTQLVTPSICSLRGAITGHEGNDDDHKWHMTVTSPNGAAFDPTEDVPAPLGTPDFTGDIYGVLSQRDRNINPGQTAPANRAHEAVVSTRSNKFTPKLGSVMIATWETTDVLQQPTKFTPVGLESPNHYNQWQLPNYSGALTLNMGLAPSVFPTYPGEQILFFRSFIPLKGGYGNSAIDCLVPQEWIQHFYQESAPSQTDVALIRYVNPETGRVLFEAKLHRQGFITVAKTGDSPINVPANGYFRFDSWVNPFYSLAPMGTGNGRRRNQ

SEQ ID NO: 30 - protein, 548 aa, Norovirus
MKMASNDAAPSNDGAAGLVPEINNEAMALEPVAGAAIAAPLTGQQNIIDPWIMNNFVQAPGGEFTVSPRNSPGEVLLNLELGPEINPYLAHLARMYNGYAGGFEVQVVLAGNAFTAGKIIFAAIPPNFPIDNLSAAQITMCPHVIVDVRQLEPVNLPMPDVRNNFFHYNQGSDSRLRLVAMLYTPLRANNSGDDVFTVSCRVLTRPSPDFSFNFLVPPTVESKTKPFTLPILTISEMSNSRFPVPIDSLHTSPTENIVVQCQNGRVTLDGELMGTTQLLPSQICAFRGVLTRSTSRASDQADTATPRLFNYYWHIQLANLNGTPYDPAEDIPGPLGTPDFRGKVFGVACQRNPDCTTRAHEAKVDTTAGRFTPKLGSLEISTESGDFDQNQPTRFTPVGIGVDHEADFQQWSLPDYSGQFTHNMNLAPAVAPNFPGEQLLFFRSQLPSSGGRSNGILDCLVPQEWVQHFYQESAPAQTQVALVRYVNPDTGRVLFEAKLHKLGFMTIAKNGDSPITVPPNGYFRFESWVNPFYTLAPMGTGNGRRRIQ

SEQ ID NO: 31 - protein, 540 aa, Norovirus
MKMASSDANPSDGSTANLVPEVNNEVMALEPVVGAAIAAPVAGQQNVIDPWIRNNFVQAPGGEFTVSPRNAPGEILWSAPLGPDLNPYLSHLARMYNSYAGGFEVQVILAGNAFTAGKIIFAAVPPNFPTEGLSPSQVTMFPHIIVDVRQLEPVLIPLPDVRNNFYHYNQSNDPTIKLIAMLYTPLRANNAGDDVFTVSCRVLTRPSPDFDFIFLVPPTVESRTKPFSVPILTVEEMTNSRFPIPLEKLFTGPSSAFVVQPQNGRCTTDGVLLGTTQLSPVNICTFRGDVTHIAGTQEYTMNLASQNWNNYDPTEEIPAPLGTPDFVGKIQGVLTQTTRRDGSTRGHKATVSTGSVHFTPKLGRIQFSTDTSNDFETGQNTRFTPVGVVQDGSTTHQNEPQQWVLPNYSGRDSHNVHLAPAVAPSFPGEQLLFFRSTMPGCSGYPNMNLDCLLPQEWVQHFYQEAAPAQSDVALLRFVNPDTGRVLFECKLHKSGYVTVAHTGQHDLVIPPNGYFRFDSWVNQFYTLAPMGNGTGRRRAL

SEQ ID NO: 32 - protein, 537 aa, Norovirus
MKMASSDANPSDGSTASLVPEVNNEVMALEPVVGAAIAAPVAGQQNVIDPWIRNNFVQAPGGEFTVSPRNAPGEILWSAPLGPDLNPYLSHLARMYNGYAGGFEVQVILAGNAFTAGKIIFAAVPPNFPTEGLSPSQVTMFPHIIVDVRQLEPVLIPLPDVRNNFYHYNQSNDSTIKLIAMLYTPLRANNAGDDVFTVSCRVLTRPSPDFDFIFLVPPTVESRTKPFSVPILTVEEMTNSRFPIPLEKLFTGPSSTFVVQPQNGRCTTDGVLLGTTQLSPVNICTFRGGITRIGQSESYKMNLASQNWNNYDPTEEIPAPLGTPDFKGRIRGLLTQTTKGAGSTRGHKATVLTGGSDFTPKLGTVRFDTKSIDFENNQNTKFTPVGVVQDGNNHDEPTQWVLPNYSGPDTHNVHLAPAVAPTFPGEQLLFFRSTMPGCSGYPKMELDCLLPQEWVQHFYQEAAPAQTDVALLRFVNPDTGRVLFECKLHKSGYVTVAHTGDHDLVIPPNGYFRFDSWVNQFYTLAPMGNGTGRRRAL

SEQ ID NO: 33 - protein, 540 aa, Norovirus
MKMASNDANPSDGSAANLVPEVNNEVMALEPVAGAALAAPVAGQQNVIDPWIRNNFVQAPGGEFTVSPRNAPGEILWSAPLSPDLNPYLSHLARMYNSYAGGFEVQVILAGNAFTAGKIIFAAVPPNFPIEGLSPSQVTMFPHIIVDVRQLEPVLIPLPDVRNNFYHYNQTNEPTIKLIAMLYTPLRANNAGEDVFTVSCRVLTRPSPDFDFIFLVPPTVESRTKPFTVPILTVEEMTNSRFPIPLEKLFTGPSSSFVVQPQNGRCTTDGVLLGTTQLSPVNICTFRGDVTHIAGSRNYTMNLASINWNNYDPTEEIPAPLGTPDFVGKIQGMLTQTTRGEGSTRAHRATVYTGSAPFTPKLGSVQFTTDTDNDFDANQNTKFTPVGVIQDGDTAHRNEPQQWVLPSYSGRNVQNVHLAPAVAPTFPGEQLLFFRSTMPGCSGYPNMDLDCLLPQEWVQHFYQEAAPAQSDVALLRFVNPDTGRVLFECKLHKSGYVTVAHTGQHDLVIPPNGYFRFDSWVNQFYTLAPMGNGAGRRRAL

SEQ ID NO: 34 - protein, 540 aa, Norovirus
MKMASNDANPSDGSAANLVPEVNNEVMALEPVVGAAIAAPVAGQQNVIDPWIRNNFVQAPGGEFTVSPRNAPGEILWSAPLGPDLNPYLSHLARMYNGYAGGFEVQVILAGNAFTAGKIIFAAVPPNFPTEGLSPSQVTMFPHIIVDVRQLEPVLIPLPDVRNNFYHYNQSNDSTIKLIAMLYTPLRANNAGDDVFTVSCRVLTRPSPDFDFIFLVPPTVESRSKPFSVPVLTVEEMTNSRFPATLDKLFTGPSSTFVVQPQNGRCMIDGVLLGTTQLSPVNICTFRGDVTHLRDSPIYTMNLASPNWNNYDSTEEIPAPLGTPDFVGKIQGVLTQTTKGEGSTRGHRATVYVGSANYTPKLGKVQFETNTTNDLYAHQNTKFTPVGVVQGGESAHRSEPQQWVLPGYSGRDTPNVHLAPAVAPTFPGEQLLFFRSTIPGCGGHPNMDLDCLLPQEWVQHFYQEAAPAQSDVALLRFVNPDTSRVLFECKLHKSGYVTVAHTGQHDLVIPPNGYFRFDSWVNQFYTLAPMGNGTGRKRAI

SEQ ID NO: 35 - protein, 539 aa, Norovirus
MKMASSDANPSDGSAANLVPEVNNEVMALEPVVGAAIAAPVAGQQNVIDPWIRNNFVQAPGGEFTVSPRNAPGEILWSAPLGPDLNPYLSHLARMYNGYAGGFEVQVILAGNAFTAGKIIFAAVPPTFPTEGLSPSQVTMFPHIIVDVRQLEPVLIPLPDVRNNFYHYNQSNDSTIKLIAMLYTPLRANNPGDDVFTVSCRVLTRPSPDFDFIFLVPPTVESRTKPFSVPILTVGEMTNSRFPINLERLFTGPSSANVVQPQNGRCTIDGELLGTTQLSSVNICTFRGDVTHIGSTHHWTMNLASPNWNNYDPTEETPAPLGTPDFVGKIHGMLTQTTQGNGSTRGHRATVYVGSAEFTPKLGKVQFKTETDHDLAIRQNTKFTPVGVIQESDHHRDEPQQWRLPNYSGANTFNVHLAPAVAPNFPGEQLLFFRSTLPGCGGHPNMDLDCLLPQEWVQHFYQEAAPAQSDVALLRFVNPDTSRVLFECKLHKSGYVTVAHTGQYDLVLPSNGYFRFDSWVNQFYTLAPMGNGTGRRRAL

SEQ ID NO: 36 - protein, 539 aa, Norovirus
MKMASNDASPSDGSAANLVPEVNNEVMALEPVVGAAIAAPVAGQQNVIDPWIRNNFVQAPGGEFTVSPRNAPGEILWSAPLGPDLNPYLSHLARMYNGYAGGFEVQVILAGNAFTAGKIIFAAVPPNFPTEGLSPSQVTMFPHIVVDVRQLEPVLIPLPDVRNNFYHYNQSKDPTIKLIAMLYTPLRANNAGEDVFTVSCRVLTRPSPDFDFIFLVPPTVESRSKPFTVPILTVEEMTNSRFPIPLEKLFTGPSGAFVVQPQNGRCTTDGVLLGTTQLSPVNICTFRGDLTHFTGTSEYAMNLASQNWDNYDPTEEIPAPLGAPDFVGKIRGMLTQTTRRDGSTRGHRATLSTGSAHFTPKLGNIRFSTDTNNDFEAGQNTKFTPVGVFQEGDNHQNEPQQWVLPNYSGATAHNVHLAPAVAPAFPGEQLLFFRSTMPGCGGYPNMNLDCLLPQEWVQHFYQEAAPAQSDVALLRFVNPDTSRVLFECKLHKSGYVTVAHTGQHDLVIPPNGYFRFDSWVNQFYTLAPMGNGTGRRRAL

SEQ ID NO: 37 - protein, 539 aa, Norovirus
MKMASSDANPSDGSTANLVPEANNEVMALEPVVGAAIAAPVAGQQNVIDPWIRNNFVQAPGGEFTVSPRNAPGEILWSAPLGPDLNPYLSHLSRMYNGYAGGFEVQVILAGNAFAAGKIIFAAVPPNFPTEGLSPSQVTMFPHLIVDVRQLEPVMIPLPDIRNNFYHYNQSNDPTIKLIAMLYTPLRANNVGDDVFTVSCRVLTRPSPDFDFIFLVPPTVESKTNPFSVPILTIEEMTNSRFPIPLEKLFTGPSSALVVQPQNGRCTTDGVLLGTTQLSPVNICTFRGDVTHTTKTHTYQMNLAAQNWNSYDPTEEIPAPLGTPDFVGKIQGVLTQTTKGNGSTRAHKATVYTGSAEFTPKLGRIQLFTDTDNDLEANQNTKFTPVGVIQDGDTHQNEPQQWVLPSYSGRNNHNVHLAPAVAPTFPGEQLLFFRSTMPGCSGYPNMNLDCLLPQEWVQYFYQEAAPAQSDVALLRFVNPDTGRVLFECKLHKSGYVTVAHTGHHDLFIPPNGYFRFDSWVSPFYTLAPMGNGTGRRRAL

SEQ ID NO: 38 - protein, 538 aa, Norovirus
MKMASSDANPSDGSAANLVPEVNNEVMALEPVVGAAIAAPVAGQQNVIDPWIRNNFVQAPGGEFTISPRNAPGEILWSAPLGPDLNPYLSHLARMYNGYAGGFEVQVVLAGNAFTAGKIIFAAVPPNFPTEGLSPSQVTMFPHIIVDVRQLEPVLIPLPDVRNNFYHYNQSKDSTIKLIAMLYTPLRANNAGDDVFTVSCRVLTRPSPDFDFIFLVPPTVESRTKPFSVPVLTVEEMTNSRFPIPLEKLFTGPSSAFVVQPQNGRCTTDGVLLGTTQLSAVNICTFRGDVTHVAGDTFAMNLASLNWNNYDPTEETPAPLGTPDFVGRIHGMLTQTTRSDGATRAHKATVSTGGADFTPKLGSVRYSTDTSSDLEVRENTKFTPIGVLHSSGGHRAEPDQWRLPEYSGRNVHNVHLAPAVAPTFPGEQLLFFRSTMPGCGGYPNMDLDCLLPQEWVQHFYQEAAPAQSDVALLRFVNPDTGRVLFECKLHKSGYVTVAHTGPHDLVIPPNGYFRFDSWVNQFYTLAPMGNGTGRRRAL

SEQ ID NO: 39 - protein, 539 aa, Norovirus
MKMASSDANPSDGSAANLVPEVNNEVMALEPVVGAAIAAPVAGQQNIIDPWIRNNFVQAPGGEFTVSPRNAPGEILWSAPLGPDLNPYLSHLSRMYNGYAGGFEVQVILAGNAFTAGKVIFAAVPPNFPTEGLSPSQVTMFPHIIVDVRQLEPVLIPLPDVRNNFYHYNQSHDSTLKLIAVLYTPLRTNNAGDDVFTVSCRVLTRPSPDFDFIFLVPPTVESRTKPFTVPILTVEEMSNSRFPIPLEKLYTGPSSAFVVQPQNGRCTTDGVLLGTTQLSAVNICNFRGDVTHIVGSHETTMNLASQNWSNYDPTQKIPAPLGTPHFVGKIQGLLTQTTRAHGSTRAHKATVSTGSVHFTPKLGSVQFTTDTNNDFQTGQNTKFTPVGVIQDGDHHQNEPQQWVLPNYSGRTGHNVHLAPAVAPTFPGEQLLFFRSTMPGCSGYPNMNLDCLLPHEWVLHFYQEAAPAQSDVALLRFVNPDTGRVLFECKLHKSGYITVAHTGPFDLGIPPNGYFRFDSWVNQFYTLAPMGNGTGRRRAL

SEQ ID NO: 40 - protein, 539 aa, Norovirus
MKMASNDASPSDGSTANLVPEVNNEVMALEPVVGAAIAAPVAGQQNVIDPWIRNSSVQAPGGEFTVSPRDAPGEILWSAPLGPDLNPYLSHLARMYNGYAGGFEVQVILAGNAFTAGKIIFAAAPPNFPTEGLSPSQVTMFPHIIVGVRQLEPVLIPLPDVRNNFYHYNQSNDSTIKLIAMLYTPLRANNAGDDVFTVSCRVLTRPSPDFDFIFLVPPTVESRTKPFTVPILTVEEMTNSRFPIPLENCSRVPAVPLSSNHKMQCTTDGVLLGTTQLSPVNICTFRGDVTHIPGTRTYRMNLASQNWNNYDPTEEIPAPLGTPDFVGKIQGMLTQTTKGDGSTRGHKATVSTGSVDFTPKLGSVQFATDTDNDFETGQNTRFTPVGVIQDGSSTHRNEPQQWVLPDYSGRTVHNVHLAPAVAPTFPGEQLLFFRSTMPGCSGYPNMDLDCLLPQEWVQHFYQEAAPSQSDVALLRFVNPDTGRVLFECKLHKAGYVTVAHTGQHDLVIPPNGYFRFDSWVNQFYTLAPMGNGAGRRRAL

SEQ ID NO: 41 - protein, 539 aa, Norovirus
MKMASSDANPSDGSSANLVPEVNNEVMALEPVVGAAIAAPVAGQQNIIDPWIRNNFVQAPGGEFTVSPRNAPGEILWSAPLSPDLNPYLSHLSRMYNGYAGGFEVQVILAGNAFTAGKIVFAAVPPNFPTEGLSPSQVTMFPHIIVDVRQLEPVLIPLPDVRNNFYHYNQANDSTLKLIAMLYTPLRANNAGDDVFTVSCRVLTRPSPDFDFIFLVPPTVESRTKPFTVPVLTVEEMTNSRFPIPLERLFTGPSTAFVVQPQNGRCTTDGVLLGTTQLSAVNICNFRGEVNHIAGTHDYTMRLTSQNWNNYDPTEEIPAPLGTPDFVGRIQGVLTQTTRSDGSTRSHKATVSTGSVHFTPKLGSVQFTTDTTNDLNAGQNTKFTPVGVEQTSGDHQSEPQQWTLPNYSGTPNHNVHLAPAVAPTFPGEQLLFFRSTLPGCGGYPNMNLDCLLPQEWVLHFYQEAAPAQSDVALLRFVNPDTGRVLFECKLHRSGFITVAHSGSHDLVIPPNGYFRFDSWVNQFYTLAPMGNGSGRRRVV

SEQ ID NO: 42 - protein, 540 aa, Norovirus
MKMASNDATPSNDGAAGLVPESNNEAMALEPVVGASLAAPVTGQTNIIDPWIRTNFVQAPNGEFTVSPRNSPGEILVNLELGPELNPYLAHLARMYNGYAGGMEVQVMLAGNAFTAGKIIFAAVPPYFPVENLSPSQITMFPHVIIDVRTLEPVLLPMPDVRSTLFHFNQKDEPKMRLVAMLYTPLRSNGSGDDVFTVSCRILTRPSPEFDFTYLVPPTVESKTKPFTLPVLTLGELSNSRFPLSIDEMVTSPNESIVVQPQNGRVTLDGELLGTTQLQACNICSIRGKVTGQVPNEQHMWNLQITNLNGTQFDPTDDVPAPLGVPDFAGEVFGVLSQRNRGESNPANRAHDAVVATYSDKYTPKLGLVQIGTWNTNDVENQPTKFTPIGLNEVANGHRFEQWTLPRYSGALTLNMNLAPAVAPLFPGERLLFFRSYVPLKGGFGNPAIDCLVPQEWVQHFYQESAPSLGDVALVRYVNPDTGRVLFEAKLHKGGFLTVSSTSTGPVVVPANGYFRFDSWVNQFYSLAPMGTGNGRRRFQ

SEQ ID NO: 43 - protein, 547 aa, Norovirus
MKMASNDAAPSNDGAANLVPEANNEVMALEPVAGASIAAPVVGQQNIIDPWIRENFVQAPQGEFTVSPRNSPGEMLLNLELGPELNPYLSHLSRMYNGYAGGMQVQVVLAGNAFTAGKIIFAAVPPHFPVKNISAAQITMCPHVIVDVRQLEPVLLPLPDIRNRFFHYNQENTPRMRLVAMLYTPLRANSGEDVFTVSCRVLTRPAPDFEFTFLVPPTVESKTKPFTLPILTLGELSNSRFPAPIDMLYTDPNEGIVVQPQNGRCTLDGTLQGTTQLVPTQICAFRGTLIGQTSRSSDSTDSAPRRRDHPLHVQLKNLDGTQYDPTDEVPAVLGAIDFKGTVFGVASQRDVSGQQVGATRAHEVHINTTDPRYTPKLGSILIHSESDDFVTGQPVRFTPIGMGDNDWHQWELPDYSGHLTLNMNLAPAVAPAFPGERILFFRSMVPSAGGYGSGQIDCLIPQEWVQHFYQEAAPSQSAVALIRYVNPDTGRNIFEAKLHREGFITVANSGNNPIVVPHNGYFRFEAWVNQFYTLTPMGTGQGRRRNQ

SEQ ID NO: 44 - protein, 540 aa, Norovirus
MKMASNDAAPSNDGAAGLVPEINNEVMPLEPVAGASLATPVVGQQNIIDPWIRNNFVQAPAGEFTVSPRNSPGEILLDLELGPELNPYLAHLARMYNGHAGGMEVQIVLAGNAFTAGKIIFAAIPPGFPYENLSPSQITMCPHVIIDVRQLEPVLLPMPDIRNNFFHYNQGNDPKLRLIAMLYTPLRANNSGDDVFTVSCRVLTKPSPDFEFTFLVPPTVESKTKQFTLPILKISEMTNSRFPVPVEMMYTARNENQVVQPQNGRVTLDGELLGTTPLLAVNICKFKGEVIAKNGDVRSYRMDMEITNTDGTPIDPTEDTPGPIGSPDFQGILFGVASQRNKNEQNPATRAHEANINTGGDQYAPKLAQVKFFSESQDFEVHQPTVFTPVGVAGDTSHPFRQWVLPRYGGHLTNNTHLAPAVAPLFPGEQILFFRSQIPSSGGHELGYMDCLVPQEWVQHFYQEAATAQSEVALIRFINPDTGRVLFEAKLHKQGFITVAHTGDNPIVMPPNGYFRFEAWVNQFYSLAPVGTGNGRRRIQ

SEQ ID NO: 45 - protein, 537 aa, Norovirus
MKMASNDAAPSNDGAAGLVPEINHEVMAIEPVAGASLAAPVVGQLNIIDPWIRNNFVQAPAGEFTVSPRNAPGEFLLDLELGPELNPYLAHLARMYNGHAGGMEVQIVLAGNAFTAGKILFAVIPPGFPYENLSPAQLTMCPHVVVDVRQLEPILLPMPDIRNTFFHYNQSNGPKLRLVAMLYTPLRANNAGDDVFTVSCRVLTRPSPDFEFNFLVPPSVESKTKAFTLPILKISEMTNSRFPIPVDQMYTSRNENVVVQPQNGRVTLDGELQGTTTLQPVSICGFRGTLQTRLADQPNYTYQVHLENLDGSPVDPTDEVPAPLGTPDFQAQLFGVVSQRSSDNATRAHEARVNTNDPTFAPQIAQVRFKSPSHDFFDNEPIKFTPVGISVDSENSYNQWLLPRYGGHLTNNTHLAPSVSPMFPGEQILFFRSFMPGASGHTDGAIDCLLPQEWVAHFYQEAATAQTDVALIRFVNPDTGRVLFEGKLHKQGFITISNSGDHPIVMPANGYFRFEAWVNQFYSLAPVGTGSGRRRIQ

SEQ ID NO: 46 - protein, 535 aa, Norovirus
MKMASNDAAPSNDGAAGLVPEVNNETMALEPVAGASIAAPLTGQNNVIDPWIRLNFVQAPNGEFTVSPRNSPGEVLLNLELGPELNPYLAHLSRMYNGYAGGVEVQVLLAGNAFTAGKLVFAAVPPHFPLENISPGQITMFPHVIIDVRTLEPVLLPLPDVRNNFFHYNQQNEPRMRLVAMLYTPLRSNGSGDDVFTVSCRVLTRPSPDFDFNYLVPPTVESKTKPFTLPILTIGELTNSRFPVPIDELYTSPNESLVVQPQNGRCALDGELQGTTQLLPTAICSFRGRINQKVSGENHVWNMQITNINGTPFDPTEDVPAPLGTPDFSGKLFGVLSQRDHDNACRSHDAVIATNSAKFTPKLGAIQIGTWEQDDVHINQPTKFTPVGLFESEGFNQWTLPNYSGALTLNMGLAPPVAPTFPGEQILFFRSHIPLKGGVADPVIDCLLPQEWIQHLYQESAPSQTDVALIRFTNPDTGRVLFEAKLHRSGYITVANTGSRPIVVPANGYFRFDSWVNQFYSLAPMGTGNGRRRVQ

SEQ ID NO: 47 - protein, 528 aa, Norovirus
MKMASNDAAPSNDGAASLVPEAINETMPLEPVAGASIAAPVAGQTNIIDPWIRTNFVQAPNGEFTVSPRNSPGEILLNLELGPDLNPYLAHLSRMYNGYAGGVEVQVLLAGNAFTAGKILFAAIPPNFPVDMISPAQITMLPHLIVDVRTLEPIMIPLPDVRNVFYHFNNQPQPRMRLVAMLYTPLRSNGSGDDVFTVSCRVLTRPTPDFEFIYLVPPSVESKTKPFTLPILTISELTNSRFPIPIEQLYTAPNENNVVQCQNGRCTLDGELQGTTQLLSSAVCSYRGRTVANRGDNWDQNLLQLTYPSGASYDPTDEVPAPLGTQDFSGILYGVLTQDNVSEGTGEAKNAKGVYISTTSGKFTPKIGSIGLHSITENVHPNQQSRFTPVGVAQNENTPFQQWVLPHYAGALALNTNLAPAVAPTFPGEQLLFFRSRVPCVQGLRGQDAFIDCLLPQEWVNHFYQEAAPSQADVALIRYVNPDTGRTLFEAKLHRSGFITVSHTGAYPLVVPPNGHFRFDSWVNQFYS

SEQ ID NO: 48 - protein, 536 aa, Norovirus
MKMASNDATPSDDGAAGLVPEINNEVMALEPVAGASIAAPVVGQQNIIDPWIRNNFVQAPAGEFTVSPRNSPGELLLDLELGPELNPYLAHLARMYNGHAGGMEVQIVLAGNAFTAGKILFAAIPPSFPYENLSPAQLTMCPHVIVDVRQLEPVLLPMPDIRNVFYHYNQNNSPKLRLVAMLYTPLRANNSGDDVFTVSCRVLTRPSPDFQFTFLVPPTVESKTKNFTLPVLRVSEMTNSRFPVVLDQMYTSRNENIIVQPQNGRCTTDGELLGTTTLQSVSICNFRGTMQAKLNEQPRYQLQLTNLDGSPIDPTDDMPAPLGTPDFQAMLYGVASQRSSRDNATRAHDAQIDTAGDTFAPKIGQVRFKSSSDDFDLHDPTKFTPIGVNVDDQHPFRQWSLPNYGGHLALNNHLAPAVTPLFPGEQILFFRSHIPSAGGHTDGAIDCLLPQEWIEHFYQEAAPSQSDIALVRFINPDTGRVLLEAKLHKQGFLTVAASGDHPIVMPTNGYFRFEAWVNPFYTLAPVGTGSGRRRIQ

SEQ ID NO: 49 - protein, 538 aa, Norovirus
MKMASNDAAPSNDGAAGLVPEGNNETLPLEPVAGAAIAAPVTGQNNIIDPWIRTNFVQAPNGEFTVSPRNSPGEILLNLELGPDLNPYLAHLSRMYNGYAGGVEVQVLLAGNAFTAGKILFAAVPPNFPVEFLSPAQITMLPHIIVDVRTLEPIMIPLPDVRNTFFHYNNQPNSRMRLVAMLYTPLRSNGSGDDVFTVSCRVLTRPTPDFEFTYLVPPSVESKTKPFSLPILTLSELTNSRFPVPIDSLFTAQNNVLQVQCQNGRCTLDGELQGTTQLLPSGICAFRGRVTAETDNPDKWHMQLQNLNGTTYDPTDDVPAPLGTPDFKGVVFGVASQRNVGNDAPGSTRAHEAVISTYSPKFVPKLGSVNFRSNDDDFQLQPTRFTPVGINDDGNHPFRQWELPDYSGVLTLNMNLAPPVAPNFPGEQLLLFRSFVPCSGGYNQGIIDCLIPQEWIQHFYQESAPSQSDVALIRYVNPDTGRTLFEAKLHRSGYITVAHSGDYPLVVPANGYFRFDSWVNQFYSLAPMGTGNGRRRAQ

SEQ ID NO: 50 - protein, 540 aa, Norovirus
MKMASNDAAPSNDGATGLVPEINNETLPLEPVAGAAIAAPVTGQNNIIDPWIRTNFVQAPNGEFTVSPRNSPGEILLNLELGPDLNPYLAHLSRMYNGYAGGVEVQVLLAGNAFTAGKILFAAVPPNFPVEFLSPAQITMLPHLIVDVRTLEPIMIPLPDVRNTFFHYNNQPANRMRLVAMLYTPLRSNGSGDDVFTVSCRVLTRPTPDFEFTYLVPPSVESKTKPFSLPILTISELTNSRFPAPIDSLFTAQNNNLNVQCQNGRCTLDGELQGTTQLLPSGICAFRGRLTADVDGSHDDRWHMQLTNLNGTPFDPTEDVPAPLGTPDFTGLLFGVASQRNVGSNPNTTRAHEAVISTTSSQFVPKLGSVNFGSTSTDFQLQQPTKFTPVGIKIESGHEFDQWALPRYSGHLTLNMNLAPPIAPNFPGEQLLFFRSNVPCAGGVSDGVIDCLLPQEWIQHFYQESAPSQSDVALIRYVNPDTGRTLFEAKLHRTGYITVAHSGDYPLVVPSNGYFRFDSWVNQFYSLAPMGTGNGRRRVQ

SEQ ID NO: 51 - protein, 540 aa, Norovirus
MKMASNDAAPSNDGAAGLVPEINTETLPLEPVAGAAIAAPVTGQNNIIDPWIRNNFVQAPNGEFTVSPRNSPGEILMNLELGPDLNPYLAHLSRMYNGYAGGVEVQVLLAGNAFTAGKILFAAVPPNFPVDMLSPAQITMLPHLIVDVRTLEPIMIPLPDVRNVFYHFNNQPAPRMRLVAMLYTPLRSNGSGDDVFTVSCRVLTRPTPDFEFTYLVPPSVESKTKPFTLPILTIGELTNSRFPAPIDQLYTSPNADVVVQPQNGRCTLDGELQGTTQLLTTAICSYRGTTSNPTSDYWDDHLLHLVHPNGATYDPTEDVPAPFGTQDFRGILYGVLTQNTQNPRDEVSNSRGIYISSTSDKFTPKLGTIGLHQVQGDTASNQQSKFTPVGIAVNQNTPFKQWELPNYSGALTLNTNLAPAVGPNFPGEQILFFRSNVPSVQGNHPTQEIDCLIPQEWISHFYQESAPSQSDVALVRYVNPDTGRTIFEAKLHRQGFITIAATGSNPVVVPPNGYFRFDSWVNQFYALAPMGTGNGRRRAQ

SEQ ID NO: 52 - protein, 541 aa, Norovirus
MKMASNDAAPSNDGAAGLVPEINTEVMALEPVAGGAIAAPLTGQTNIIDPWIRNNFVQAPNGEFTISPRNSPGEILLNMELGPELNPFLAHLSRMYNGFAGGMEVQVLMAGNAFTAGKVIFAAIPPHFPVENLSPPQITMFPHIIIDVRTLEPVLLPMPDVRNQFFHYNQVNEPRMRLVAMLYTPLRSNGSTEDVFTVSCRVLTRPSPDFEFNYLVPPTVESRTKPFTLPILTIGEMTNSRFPAPIDMLYTSPNDNVVVQPQNGRCTLDGELQGSTQLVPANVCAFKGKITARIVDQAAHQWHMQIDNPNGTLFDPTEDVPAPLGTPDFKAKIFGVISQRNDYNDGSQGPANRAHDAVVPTTSAKFTPKLGSILVGTWENNDIETQPSKFTPVGLLEMNDFNQWSLPNYSGALTLNMGLAPAVFPTFPGEQILFFRSFIPLKGGHGNPAIDCLLPQEWIQHFYQESAPSQTSVALIRYVNPDTGRVLFEGKLHRQGFITIAKSGDGPIVVPPNGYFRFDSWVNQFYSLAPMGNGNGRRRIQ

SEQ ID NO: 53 - protein, 542 aa, Norovirus
MKMASNDAAPSNDGAANLVPEANKEVMALEPVAGGAIAAPLTGQTNIIDPWIMNNFVQAPNGEFTISPRNSPGEVLLNLELGPDLNPFLAHLSRMYNGYAGGVEVQVIMAGNAFTAGKVIFAAVPPHFPVDNLSPPQVTMFPHVIVDVRTFEPILLPLPDVRNSFYHYNQVNDSRMRLIAMLYTPLRSNGSSDDVFTVSCRVLTRPTPDFEFNYLVPPTVESRTKPFSVPILTIGEMTNSRFPLPIDMLYTSPTENIVVQPQNGRCTLEGELLGTTQLVTPNICALRGEIRGHEGSGDNHKWHFMVRSPNGAAFDPTEDVPAPLGTPDFIGDVFGVLSQRNRNTDSGQSGPANRSHDAVVSTRDSRFTPKLGSVMIATWETSDIQDQPTRFTPVGLENPDHYNQWQLPNYSGALTLNMGLAPSVFPTYPGEQILFFRSYIPLKGGYGDSHIDCLVPQEWIQHFYQESAPSQTDVALIRYVNPETGRVLFEAKLHRQGYITVARSGSSPINVPANGYFRFDSWVNQFYSLAPMGTGNGRRRIQ

SEQ ID NO: 54 - protein, 541 aa, Norovirus
MKMASNDAAPSNDGAAGLVPEINNEVMALEPVAGGAIAAPLTGQTNVIDPWIRTNFVQAPNGEFTISPRNSPGEVLLNMELGPELNPFLGHLSRMYNGYAGGIEVQVLMAGNAFTAGKVIFAAVPPHFPVENLSPPQVTMFPHIIVDVRTLEPILLPLPDVRNQFFHYSQVDEPKMRLVAMLYTPLRSNGSAEDVFTVSCRVLTRPSPDFEFNYLVPPTVESRTKPFTVPILTIGEMSNSRFPAPIDMLYTSPNDNQNVQPQNGRCTLDGELQGTTQLVPSGVCAFRGRITGHEGSEQNQWHMQLTNLNGTPFDPTEDIPAPLGTPDFKGEIFGFISQRNAQNDPGQSQPANRAHDAVVSTRAPKFTPKLGSVMIGTWVNSDIENQPSKFTPVGLNSNENFRQWELPDYSGVLTLNMGLAPVVHPTYPGEQILFFRSYIPLKGGHGNPAIDCLLPQEWIQHFYQESAPSQTDVALLRYVNPDTGRVLFEAKLHRQGYITIAKSGDGPIVVPPNGYFRFDSWVNQFYSLAPMGNGNGRRRVQ

SEQ ID NO: 55 - protein, 556 aa, Norovirus
MKMASSDAAPSTDGAGNLVPESQQEVLPLAPVAGAALAAPVVGQTNIIDPWIKENFVQAPQGEFTVSPKNSPGEILVNLELGPKLNPYLDHLSRMYNSYAGGIDVMVVLAGNAFTAGKVLIAAIPPNFPVEGVSASQATQFPHVIIDVRTLDPVRLPLPDVRSTFFHYTNDTEPKMRLVIWLYTPLRTNGSGDDSFTVSGRILTRPSQDFEFAFLIPPTVETKTTPFSVPGFSVQEMSNSRWPAAISAMVVRGNEPQVVQFQNGRAHLDGMLLGTTPVSPNYIASYRGISTGNSRSASSEADERAVGSFDVWVRLQEPDGQPYDIFGKQPAPIGTPDFKAVIVGFAARPLTSGSYANEAYVNTTASDYAPATGNMRFTVRNGGTGHISANKYWEFKSFGVEGERHTDIQYQEYELPDYSGQVASNHNLAPPVAPRMPGESLLLFQSNMPVWDDGHGESTPKKIHCLLPQEFIGHFFDRQAPSLGDAALLRYVNQETNRVLFECKLYRDGYITVAASSGLLDFPLDGFFRFDSWVSSFYILSPVGSGQGRRGRVRFQ

SEQ ID NO: 56 - protein, 554 aa, Norovirus
MKMASNDAPPSSDGAGNLVPESHQEVLPLAPVAGAELAAPVVGQTNIIDPWIKENFVQAPQGEFTVSPKNAPGEILVNLELGPNLNPYLEHLSRMYNAYAGGIEVEIILAGNAFTAGKILIAAVPPNFPVESVSASQATQFPHAIVDVRTLEPVRLPLPDVRSNFFHYTTKDEPKMRLVIWLYTPLRTNGSGDDSFTVSGRLLTRPSMDFQFSFLVPPTVETKTVLFTVPGLTPQEMSNSRWPAQISGMVVRGNEPQVVQFQNGRCHTDGTLLGTTTVSEQCIAGFVGTSTNTRSATGSTTETRTGDTDLWLRLEEPNGQPYDIFGDQPAPLGTPDFRAVIVGFASRPQTQGSYMNEAYVNTVDSHFAPATGNTKIILRRGGTGHVGGGHLWKFRPFGVEGGEGRVSYQEYVLPNYSGATASNHNLAPPVAPRMPGELLLLFESDMPVWDDGHGAAPAQKIHCLLPQQFITHFFDSQAPALAEAALLRYVHPDSSRVLFETKLYREGFMVVSAPTGRFDFPLDGYFRFDSWVNSFYVLSPVGSGQGRRGRSKVV

SEQ ID NO: 57 - protein, 6 aa, artificial
  sequence stretch with variant amino acid residue
  VARIANT (4)..(4): Leu or Val
AALXHY

SEQ ID NO: 58 - protein, 6 aa, Artificial Sequence
  sequence stretch with variant amino acid residue
  VARIANT (4)..(4): Leu or Val
  VARIANT (5)..(5): Arg or Lys
AALXXY

SEQ ID NO: 59 - protein, 8 aa, Artificial Sequence
  sequence stretch with variant amino acid residue
  variant (4)..(4): Leu or Val
  variant (7)..(7): Val, Leu or Ile
AALXHYXD

SEQ ID NO: 60 - protein, 8 aa, Artificial Sequence
  sequence stretch with variant amino acid residue
  variant (4)..(4): Leu or Val
  variant (5)..(5): Arg or Lys
  variant (7)..(7): Val or Leu or Ile
AALXXYXD

SEQ ID NO: 61 - protein, 5 aa, Artificial Sequence
  sequence stretch with variant amino acid residue
  VARIANT (4)..(4): Leu or Val
AALXH